European Patent Application EP 4 353 319 A2, published April 17, 2024. Title: METHODS OF ADOPTIVE CELL THERAPY. Applicant: ATOSSA GENETICS INC. The sequence listing filed with the application follows.

SEQUENCE LISTING (11 sequences)

SEQ ID NO: 1 - DNA, 7217 bp, synthetic construct
  misc_feature 1..7217: note = synthetic
  source 1..7217: mol_type = other DNA
ggccgcattcgtgccggtcttcctgccagcgaagcccaccacgacgccagcgccgcgaccaccaacaccggcgcccaccatcgcgtcgcagcccctgtccctgcgcccagaggcgtgccggccagcggcggggggcgcagtgcacacgagggggctggacttcgcctgtgatatctacatctgggcgcccttggccgggacttgtggggtccttctcctgtcactggttatcaccctttactgcaaccacaggaacaggagtaagaggagcaggctcctgcacagtgactacatgaacatgactccccgccgccccgggcccacccgcaagcattaccagccctatgccccaccacgcgacttcgcagcctatcgctcccgtttctctgttgttaaacggggcagaaagaagctcctgtatatattcaaacaaccatttatgagaccagtacaaactactcaagaggaagatggctgtagctgccgatttccagaagaagaagaaggaggatgtgaactgagagtgaagttcagcaggagcgcagacgcccccgcgtaccagcagggccagaaccagctctataacgagctcaatctaggacgaagagaggagtacgatgttttggacaagagacgtggccgggaccctgagatggggggaaagccgagaaggaagaaccctcaggaaggcctgtacaatgaactgcagaaagataagatggcggaggcctacagtgagattgggatgaaaggcgagcgccggaggggcaaggggcacgatggcctttaccagggtctcagtacagccaccaaggacacctacgacgcccttcacatgcaggccctgccccctcgctaaggatccgataaaataaaagattttatttagtctccagaaaaaggggggaatgaaagaccccacctgtaggtttggcaagctagcttaagtaacgccattttgcaaggcatggaaaatacataactgagaatagagaagttcagatcaaggttaggaacagagagacagcagaatatgggccaaacaggatatctgtggtaagcagttcctgccccggctcagggccaagaacagatggtccccagatgcggtcccgccctcagcagtttctagagaaccatcagatgtttccagggtgccccaaggacctgaaaatgaccctgtgccttatttgaactaaccaatcagttcgcttctcgcttctgttcgcgcgcttctgctccccgagctcaataaaagagcccacaacccctcactcggcgcgccagtcctccgatagactgcgtcgcccgggtacccgtgtatccaataaaccctcttgcagttgcatccgacttgtggtctcgctgttccttgggagggtctcctctgagtgattgactacccgtcagcgggggtctttcatgggtaacagtttcttgaagttggagaacaacattctgagggtaggagtcgaatattaagtaatcctgactcaattagccactgttttgaatccacatactccaatactcctgaaatccatcgatggagttcattatggacagcgcagaaagagctggggagaattgtgaaattgttatccgctcacaattccacacaacatacgagccggaagcataaagtgtaaagcctggggtgcctaatgagtgagctaactcacattaattgcgttgcgctcactgcccgctttccagtcgggaaacctgtcgtgccagctgcattaatgaatcggccaacgcgcggggagaggcggtttgcgtattgggcgctcttccgcttcctcgctcactgactcgctgcgctcggtcgttcggctgcggcgagcggtatcagctcactcaaaggcggtaatacggttatccacagaatcaggggataacgcaggaaagaacatgtgagcaaaaggccagcaaaaggccaggaaccgtaaaaaggccgcgttgctggcgtttttccataggctccgcccccctgacgagcatcacaaaaatcgacgctcaagtcagaggtggcgaaacccgacaggactataaagataccaggcgtttccccctggaagctccctcgtgcgctctcctgttccgaccctgccgcttaccggatacctgtccgcctttctcccttcgggaagcgtggcgctttctcatagctcacgctgtaggtatctcagttcggtgtaggtcgttcgctccaagctgggctgtgtgcacgaaccccccgttcagcccgaccgctgcgccttatccggtaactatcgtcttgagtccaacccggtaagacacgacttatcgccactggcagcagccactggtaacaggattagcagagcgaggtatgtaggcggtgctacagagttcttgaagtggtggcctaactacggctacactagaaggacagtatttggtatctgcgctctgctgaagccagttaccttcggaaaaagagttggtagctcttgatccggcaaacaaaccaccgctggtagcggtggtttttttgtttgcaagcagcagattacgcgcagaaaaaaaggatctcaagaagatcctttgatcttttctacggggtctgacgctcagtggaacgaaaactcacgttaagggattttggtcatgagattatcaaaaaggatcttcacctagatccttttaaattaaaaatgaagttttaaatcaatctaaagtatatatgagtaaacttggtctgacagttaccaatgcttaatcagtgaggcacctatctcagcgatctgtctatttcgttcatccatagttgcctgactccccgtcgtgtagataactacgatacgggagggcttaccatctggccccagtgctgcaatgataccgcgagacccacgctcaccggctccagatttatcagcaataaaccagccagccggaagggccgagcgcagaagtggtcctgcaactttatccgcctccatccagtctattaattgttgccgggaagctagagtaagtagttcgccagttaatagtttgcgcaacgttgttgccattgctacaggcatcgtggtgtcacgctcgtcgtttggtatggcttcattcagctccggttcccaacgatcaaggcgagttacatgatcccccatgttgtgcaaaaaagcggttagctccttcggtcctccgatcgttgtcagaagtaagttggccgcagtgttatcactcatggttatggcagcactgcataattctcttactgtcatgccatccgtaagatgcttttctgtgactggtgagtactcaaccaagtcattctgagaatagtgtatgcggcgaccgagttgctcttgcccggcgtcaatacgggataataccgcgccacatagcagaactttaaaagtgctcatcattggaaaacgttcttcggggcgaaaactctcaaggatcttaccgctgttgagatccagttcgatgtaacccactcgtgcacccaactgatcttcagcatcttttactttcaccagcgtttctgggtgagcaaaaacaggaaggcaaaatgccgcaaaaaagggaataagggcgacacggaaatgttgaatactcatactcttcctttttcaatattattgaagcatttatcagggttattgtctcatgagcggatacatatttgaatgtatttagaaaaataaacaaataggggttccgcgcacatttccccgaaaagtgccacctgacgtctaagaaaccattattatcatgacattaacctataaaaataggcgtatcacgaggccctttcgtctcgcgcgtttcggtgatgacggtgaaaacctctgacacatgcagctcccggagacggtcacagcttgtctgtaagcggatgccgggagcagacaagcccgtcagggcgcgtcagcgggtgttggcgggtgtcggggctggcttaactatgcggcatcagagcagattgtactgagagtgcaccatatgcggtgtgaaataccgcacagatgcgtaaggagaaaataccgcatcaggcgccattcgccattcaggctgcgcaactgttgggaagggcgatcggtgcgggcctcttcgctattacgccagctggcgaaagggggatgtgctgcaaggcgattaagttgggtaacgccagggttttcccagtcacgacgttgtaaaacgacggccagtgccacgctctcccttatgcgactcctgcattaggaagcagcccagtagtaggttgaggccgttgagcaccgccgccgcaaggaatggtgcatgcaaggagatggcgcccaacagtcccccggccacggggcctgccaccatacccacgccgaaacaagcgctcatgagcccgaagtggcgagcccgatcttccccatcggtgatgtcggcgatataggcgccagcaaccgcacctgtggcgccggtgatgccggccacgatgcgtccggcgtagaggcgatttaaagacaggatatcagtggtccaggctctagttttgactcaacaatatcaccagctgaagcctatagagtacgagccatagataaaataaaagattttatttagtctccagaaaaaggggggaatgaaagaccccacctgtaggtttggcaagctagcttaagtaacgccattttgcaaggcatggaaaatacataactgagaatagagaagttcagatcaaggttaggaacagagagacagcagaatatgggccaaacaggatatctgtggtaagcagttcctgccccggctcagggccaagaacagatggtccccagatgcggtcccgccctcagcagtttctagagaaccatcagatgtttccagggtgccccaaggacctgaaaatgaccctgtgccttatttgaactaaccaatcagttcgcttctcgcttctgttcgcgcgcttctgctccccgagctcaataaaagagcccacaacccctcactcggcgcgccagtcctccgatagactgcgtcgcccgggtacccgtattcccaataaagcctcttgctgtttgcatccgaatcgtggactcgctgatccttgggagggtctcctcagattgattgactgcccacctcgggggtctttcatttggaggttccaccgagatttggagacccctgcctagggaccaccgacccccccgccgggaggtaagctggccagcggtcgtttcgtgtctgtctctgtctttgtgcgtgtttgtgccggcatctaatgtttgcgcctgcgtctgtactagttagctaactagctctgtatctggcggacccgtggtggaactgacgagttcggaacacccggccgcaaccctgggagacgtcccagggacttcgggggccgtttttgtggcccgacctgagtccaaaaatcccgatcgttttggactctttggtgcaccccccttagaggagggatatgtggttctggtaggagacgagaacctaaaacagttcccgcctccgtctgaatttttgctttcggtttgggaccgaagccgcgccgcgcgtcttgtctgctgcagcatcgttctgtgttgtctctgtctgactgtgtttctgtatttgtctgagaatatgggcccgggctagcctgttaccactcccttaagtttgaccttaggtcactggaaagatgtcgagcggatcgctcacaaccagtcggtagatgtcaagaagagacgttgggttaccttctgctctgcagaatggccaacctttaacgtcggatggccgcgagacggcacctttaaccgagacctcatcacccaggttaagatcaaggtcttttcacctggcccgcatggacacccagaccaggtcccctacatcgtgacctgggaagccttggcttttgacccccctccctgggtcaagccctttgtacaccctaagcctccgcctcctcttcctccatccgccccgtctctcccccttgaacctcctcgttcgaccccgcctcgatcctccctttatccagccctcactccttctctaggcgcccccatatggccatatgagatcttatatggggcacccccgccccttgtaaacttccctgaccctgacatgacaagagttactaacagcccctctctccaagctcacttacaggctctctacttagtccagcacgaagtctggagacctctggcggcagcctaccaagaacaactggaccgaccggtggtacctcacccttaccgagtcggcgacacagtgtgggtccgccgacaccagactaagaacctagaacctcgctggaaaggaccttacacagtcctgctgaccacccccaccgccctcaaagtagacggcatcgcagcttggatacacgccgcccacgtgaaggctgccgaccccgggggtggaccatcctctagactgctcgaggccgccatggattttcaggtgcagattttcagcttcctgctaatcagtgcctcagtcataatgtccagaggagatatccagatgacccagtccccgagctccctgtccgcctctgtgggcgatagggtcaccatcacctgccgtgccagtcaggatgtgaatactgctgtagcctggtatcaacagaaaccaggaaaagctccgaaactactgatttactcggcatccttcctttattctggagtcccttctcgcttctctggatctagatctgggacggatttcactctgaccatcagcagtctgcagccggaagacttcgcaacttattactgtcagcaacattatactactcctcccacgttcggacagggtaccaaggtggagatcaaacgcactgggtctacatctggatctgggaagccgggttctggtgagggttctgaggttcagctggtggagtctggcggtggcctggtgcagccagggggctcactccgtttgtcctgtgcagcttctggcttcaacattaaagacacctatatacactgggtgcgtcaggccccgggtaagggcctggaatgggttgcaaggatttatcctacgaatggttatactagatatgccgatagcgtcaagggccgtttcactataagcgcagacacatccaaaaacacagcctacctgcagatgaacagcctgcgtgctgaggacactgccgtctattattgttctagatggggaggggacggcttctatgctatggacgtgtggggtcaaggaaccctggtcaccgtctcctcggc

SEQ ID NO: 2 - DNA, 1479 bp, synthetic construct
  misc_feature 1..1479: note = synthetic
  source 1..1479: mol_type = other DNA
atggccctgcctgtgacagccctgctgctgcctctggctctgctgctgcatgccgctagacctggatcccaggtgcagctgaaagagtccggcggaggactggtgcagcctggcggatctctgaagctgagctgtgctgccagcggcttcaccttcagcagctacggcatgagctgggtgcgacagaccgccgacaagagactggaactggtggctaccaccaacaacaacggcggcgtgacctactaccccgacagcgtgaagggcagattcaccatctccagagacaacgccaagaacaccctgtacctgcagatgagcagcctgcagagcgaggacaccgccatgtactactgcgccagatacggctactacgccatggattactggggccagggcatcagcgtgaccgtgtctagcggaggcggcggatctggcggagggggatctagtggcggaggctctgacgtgctgatgacccagacacctctgagcctgccagtgtccctgggcgaccaggccagcatcagctgtagaagcagccagagcatcgtgcacagcaacggcaacacctacctggaatggtatctgcagaagcccggccagagccccaagctgctgatctacaaggtgtccaacagattcagcggcgtgcccgacagattctccggcagcggctctggcaccgacttcaccgtgaagatctccagggtggaagccgaggacctgggcgtgtactactgttttcaaggcagccacgtgccctacaccttcggcggaggcaccaagctggaaatcaaggctagctccggaaccacgacgccagcgccgcgaccaccaacaccggcgcccaccatcgcgtcgcagcccctgtccctgcgcccagaggcgtgccggccagcggcggggggcgcagtgcacacgagggggctggacttcgcctgtgatatctacatctgggcgcccaggccgggacttgtggggtccactcctgtcactggttatcaccattactgcaaacggggcagaaagaaactcctgtatatattcaaacaaccatttatgagaccagtacaaactactcaagaggaagatggctgtagctgccgatttccagaagaagaagaaggaggatgtgaactgagagtgaagttcagcaggagcgcagacgcccccgcgtacaagcagggccagaaccagctctataacgagctcaatctaggacgaagagaggagtacgatgttttggacaagagacgtggccgggaccctgagatggggggaaagccgagaaggaagaaccctcaggaaggcctgtacaatgaactgcagaaagataagatggcggaggcctacagtgagattgggatgaaaggcgagcgccggaggggcaaggggcacgatggcctttaccagggtctcagtacagccaccaaggacacctacgacgcccttcacatgcaggccctgccccctcgc

SEQ ID NO: 3 - DNA, 63 bp, synthetic construct
  misc_feature 1..63: note = synthetic
  source 1..63: mol_type = other DNA
atggccctgcctgtgacagccctgctgctgcctctggctctgctgctgcatgccgctagacct

SEQ ID NO: 4 - DNA, 732 bp, synthetic construct
  misc_feature 1..732: note = synthetic
  source 1..732: mol_type = other DNA
caggtgcagctgaaagagtccggcggaggactggtgcagcctggcggatctctgaagctgagctgtgctgccagcggcttcaccttcagcagctacggcatgagctgggtgcgacagaccgccgacaagagactggaactggtggctaccaccaacaacaacggcggcgtgacctactaccccgacagcgtgaagggcagattcaccatctccagagacaacgccaagaacaccctgtacctgcagatgagcagcctgcagagcgaggacaccgccatgtactactgcgccagatacggctactacgccatggattactggggccagggcatcagcgtgaccgtgtctagcggaggcggcggatctggcggagggggatctagtggcggaggctctgacgtgctgatgacccagacacctctgagcctgccagtgtccctgggcgaccaggccagcatcagctgtagaagcagccagagcatcgtgcacagcaacggcaacacctacctggaatggtatctgcagaagcccggccagagccccaagctgctgatctacaaggtgtccaacagattcagcggcgtgcccgacagattctccggcagcggctctggcaccgacttcaccgtgaagatctccagggtggaagccgaggacctgggcgtgtactactgttttcaaggcagccacgtgccctacaccttcggcggaggcaccaagctggaaatcaag

SEQ ID NO: 5 - DNA, 135 bp, synthetic construct
  misc_feature 1..135: note = synthetic
  source 1..135: mol_type = other DNA
accacgacgccagcgccgcgaccaccaacaccggcgcccaccatcgcgtcgcagcccctgtccctgcgcccagaggcgtgccggccagcggcggggggcgcagtgcacacgagggggctggacttcgcctgtgat

SEQ ID NO: 6 - DNA, 72 bp, synthetic construct
  misc_feature 1..72: note = synthetic
  source 1..72: mol_type = other DNA
atctacatctgggcgcccttggccgggacttgtggggtccttctcctgtcactggttatcaccctttactgc

SEQ ID NO: 7 - DNA, 126 bp, synthetic construct
  misc_feature 1..126: note = synthetic
  source 1..126: mol_type = other DNA
aaacggggcagaaagaaactcctgtatatattcaaacaaccatttatgagaccagtacaaactactcaagaggaagatggctgtagctgccgatttccagaagaagaagaaggaggatgtgaactg

SEQ ID NO: 8 - DNA, 336 bp, synthetic construct
  misc_feature 1..336: note = synthetic
  source 1..336: mol_type = other DNA
agagtgaagttcagcaggagcgcagacgcccccgcgtacaagcagggccagaaccagctctataacgagctcaatctaggacgaagagaggagtacgatgttttggacaagagacgtggccgggaccctgagatggggggaaagccgagaaggaagaaccctcaggaaggcctgtacaatgaactgcagaaagataagatggcggaggcctacagtgagattgggatgaaaggcgagcgccggaggggcaaggggcacgatggcctttaccagggtctcagtacagccaccaaggacacctacgacgcccttcacatgcaggccctgccccctcgc

SEQ ID NO: 9 - DNA, 25 bp, synthetic construct
  misc_feature 1..25: note = synthetic
  source 1..25: mol_type = other DNA
tgccgatttccagaagaagaagaag

SEQ ID NO: 10 - DNA, 17 bp, synthetic construct
  misc_feature 1..17: note = synthetic
  source 1..17: mol_type = other DNA
tgcgctcctgctgaact

SEQ ID NO: 11 - DNA, 19 bp, synthetic construct
  misc_feature 1..19: note = synthetic
  source 1..19: mol_type = other DNA
cactctcagttcacatcct